European Patent Application EP 4 725 952 A1, published April 15, 2026. Title: COMPOUNDS COMPRISING NON-CANONICAL AMINO ACIDS AND USES THEREOF. Applicant: ETH Zurich. Application EP. The sequence listing filed with the application follows.

SEQUENCE LISTING (64 sequences)

SEQ ID NO: 1 - protein, 543 aa, Escherichia coli
MTNITKRSLVAAGVLAALMAGNVALAADVPAGVTLAEKQTLVRNNGSEVQSLDPHKIEGVPESNISRDLFEGLLVSDLDGHPAPGVAESWDNKDAKVWTFHLRKDAKWSDGTPVTAQDFVYSWQRSVDPNTASPYASYLQYGHIAGIDEILEGKKPITDLGVKAIDDHTLEVTLSEPVPYFYKLLVHPSTSPVPKAAIEKFGEKWTQPGNIVTNGAYTLKDWVVNERIVLERSPTYWNNAKTVINQVTYLPIASEVTDVNRYRSGEIDMTNNSMPIELFQKLKKEIPDEVHVDPYLCTYYYEINNQKPPFNDVRVRTALKLGMDRDIIVNKVKAQGNMPAYGYTPPYTDGAKLTQPEWFGWSQEKRNEEAKKLLAEAGYTADKPLTINLLYNTSDLHKKLAIAASSLWKKNIGVNVKLVNQEWKTFLDTRHQGTFDVARAGWCADYNEPTSFLNTMLSNSSMNTAHYKSPAFDSIMAETLKVTDEAQRTALYTKAEQQLDKDSAIVPVYYYVNARLVKPWVGGYTGKDPLDNTYTRNMYIVKH

SEQ ID NO: 2 - protein, 419 aa, Methanosarcina barkeri
MDKKPLDVLISATGLWMSRTGTLHKIKHHEVSRSKIYIEMACGDHLVVNNSRSCRTARAFRHHKYRKTCKRCRVSDEDINNFLTRSTESKNSVKVRVVSAPKVKKAMPKSVSRAPKPLENSVSAKASTNTSRSVPSPAKSTPNSSVPASAPAPSLTRSQLDRVEALLSPEDKISLNMAKPFRELEPELVTRRKNDFQRLYTNDREDYLGKLERDITKFFVDRGFLEIKSPILIPAEYVERMGINNDTELSKQIFRVDKNLCLRPMLAPTLYNYLRKLDRILPGPIKIFEVGPCYRKESDGKEHLEEFTMVNFCQMGSGCTRENLEALIKEFLDYLEIDFEIVGDSCMVYGDTLDIMHGDLELSSAVVGPVSLDREWGIDKPWIGAGFGLERLLKVMHGFKNIKRASRSESYYNGISTNL

SEQ ID NO: 3 - protein, 419 aa, synthetic construct
MDKKPLDVLISATGLWMSRTGTLHKIKHHEVSRSKIYIEMACGDHLVVNNSRSCRTARAFRHHKYRKTCKRCRVSDEDINNFLTRSTESKNSVKVRVVSAPKVKKAMPKSVSRAPKPLENSVSAKASTNTSRSVPSPAKSTPNSSVPASAPAPSLTRSQLDRVEALLSPEDKISLNMAKPFRELEPELVTRRKNDFQRLYTNDREDYLGKLERDITKFFVDRGFLEIKSPILIPAEYVERMGINNDTELSKQIFRVDKNLCLRPMLAPTLYNYLRKLDRILPGPIKIFEVGPCYRKESDGKEHLEEFTMVNFVQMGSGCTRENLEALIKEFLDYLEIDFEIVGDSCMVYGDTLDIMHGDLELSSAVVGPVSLDREWGIDKPWIGAGFGLERLLKVMHGFKNIKRASRSESYYNGISTNL

SEQ ID NO: 4 - protein, 419 aa, synthetic construct
MDKKPLDVLISATGLWMSRTGTLHKIKHHEVSRSKIYIEMACGDHLVVNNSRSCRTARAFRHHKYRKTCKRCRVSDEDINNFLTRSTESKNSVKVRVVSAPKVKKAMPKSVSRAPKPLENSVSAKASTNTSRSVPSPAKSTPNSSVPASAPAPSLTRSQLDRVEALLSPEDKISLNMAKPFRELEPELVTRRKNDFQRLYTNDREDYLGKLERDITKFFVDRGFLEIKSPILIPAEYVERMGINNDTELSKQIFRVDKNLCLRPMLAPTLLNYLRKLDRILPGPIKIFEVGPCYRKESDGKEHLEEFTMVNFTQMGSGCTRENLEALIKEFLDYLEIDFEIVGDSCMVYGDTLDIMHGDLELSSAVVGPVSLDREWGIDKPWIGAGFGLERLLKVMHGFKNIKRASRSESYYNGISTNL

SEQ ID NO: 5 - protein, 454 aa, synthetic construct
MDKKPLNTLISATGLWMSRTGTIHKIKHHEVSRSKIYIEMACGDHLVVNNSRSSRTARALRHHKYRKTCKRCRVSDEDLNKFLTKANEDQTSVKVKVVSAPTRTKKAMPKSVARAPKPLENTEAAQAQPSGSKFSPAIPVSTQESVSVPASVSTSISSISTGATASALVKGNTNPITSMSAPVQASAPALTKSQTDRLEVLLNPKDEISLNSGKPFRELESELLSRRKKDLQQIYAEERENYLGKLEREITRFFVDRGFLEIKSPILIPLEYIERMGIDNDTELSKQIFRVDKNFCLRPMLAPNLMNYARKLDRALPDPIKIFEIGPCYRKESDGKEHLEEFTMLNFAQMGSGCTRENLESIITDFLNHLGIDFKIVGDSCMVYGDTLDVMHGDLELSSAVVGPIPLDREWGIDKPWIGAGFGLERLLKVKHDFKNIKRAARSESYYNGISTNL

SEQ ID NO: 6 - protein, 275 aa, synthetic construct
MTVKYTDAQIQRLREYGNGTYEQKVFEDLASRDAAFSKEMSVASTDNEKKIKGMIANPSRHGLTQLMNDIADALVAEGFIEVRTPIFISKDALARMTITEDKPLFKQVFWIDEKRALRPMLAPNLYSVMRDLRDHTDGPVKIFEMGSCFRKESHSGMHLEEFTMLNLVDMGPRGDATEVLKNYISVVMKAAGLPDYDLVQEESDVYKETIDVEINGQEVCSAAVGPIPLDAAHDVHEPWSGAGFGLERLLTIREKYSTVKKGGASISYLNGAKIN

SEQ ID NO: 7 - protein, 454 aa, Methanosarcina mazei
MDKKPLNTLISATGLWMSRTGTIHKIKHHEVSRSKIYIEMACGDHLVVNNSRSSRTARALRHHKYRKTCKRCRVSDEDLNKFLTKANEDQTSVKVKVVSAPTRTKKAMPKSVARAPKPLENTEAAQAQPSGSKFSPAIPVSTQESVSVPASVSTSISSISTGATASALVKGNTNPITSMSAPVQASAPALTKSQTDRLEVLLNPKDEISLNSGKPFRELESELLSRRKKDLQQIYAEERENYLGKLEREITRFFVDRGFLEIKSPILIPLEYIERMGIDNDTELSKQIFRVDKNFCLRPMLAPNLYNYLRKLDRALPDPIKIFEIGPCYRKESDGKEHLEEFTMLNFCQMGSGCTRENLESIITDFLNHLGIDFKIVGDSCMVYGDTLDVMHGDLELSSAVVGPIPLDREWGIDKPWIGAGFGLERLLKVKHDFKNIKRAARSESYYNGISTNL

SEQ ID NO: 8 - protein, 275 aa, synthetic construct
MTVKYTDAQIQRLREYGNGTYEQKVFEDLASRDAAFSKEMSVASTDNEKKIKGMIANPSRHGLTQLMNDIADALVAEGFIEVRTPIFISKDALARMTITEDKPLFKQVFWIDEKRALRPMLAPNLYSVMRDLRDHTDGPVKIFEMGSCFRKESHSGMHLEEFTMLNLVDMGPRGDATEVLKNYISVVMKAAGLPDYDLVQEESDVYKETIDVEINGQEVCSAAVGPHYLDAAHDVHEPWSGAGFGLERLLTIREKYSTVKKGGASISYLNGAKIN

SEQ ID NO: 9 - protein, 306 aa, Methanocaldococcus jannaschii
MDEFEMIKRNTSEIISEEELREVLKKDEKSAYIGFEPSGKIHLGHYLQIKKMIDLQNAGFDIIILLADLHAYLNQKGELDEIRKIGDYNKKVFEAMGLKAKYVYGSEFQLDKDYTLNVYRLALKTTLKRARRSMELIAREDENPKVAEVIYPIMQVNDIHYLGVDVAVGGMEQRKIHMLARELLPKKVVCIHNPVLTGLDGEGKMSSSKGNFIAVDDSPEEIRAKIKKAYCPAGVVEGNPIMEIAKYFLEYPLTIKRPEKFGGDLTVNSYEELESLFKNKELHPMDLKNAVAEELIKILEPIRKRL

SEQ ID NO: 10 - protein, 323 aa, Archaeoglobus fulgidus
MDITEKLRLITRNAEEVVTEEELRQLIETKEKPRAYVGYEPSGEIHLGHMMTVQKLMDLQEAGFEIIVLLADIHAYLNEKGTFEEIAEVADYNKKVFIALGLDESRAKFVLGSEYQLSRDYVLDVLKMARITTLNRARRSMDEVSRRKEDPMVSQMIYPLMQALDIAHLGVDLAVGGIDQRKIHMLARENLPRLGYSSPVCLHTPILVGLDGQKMSSSKGNYISVRDPPEEVERKIRKAYCPAGVVEENPILDIAKYHILPRFGKIVVERDAKFGGDVEYASFEELAEDFKSGQLHPLDLKIAVAKYLNMLLEDARKRLGVSV

SEQ ID NO: 11 - protein, 537 aa, Methanococcus maripaludis
MFKREEIIEMANKDFEKAWIETKDLIKAKKINESYPRIKPVFGKTHPVNDTIENLRQAYLRMGFEEYINPVIVDERDIYKQFGPEAMAVLDRCFYLAGLPRPDVGLSDEKISQIEKLGIKVSEHKESLQKILHGYKKGTLDGDDLVLEISNALEISSEMGLKILEDVFPEFKDLTAVSSKLTLRSHMTSGWFLTVSDLMNKKPLPFKLFSIDRCFRREQKEDKSHLMTYHSASCAIAGEGVDINDGKAIAEGLLSQFGFTNFKFIPDEKKSKYYTPETQTEVYAYHPKLKEWLEVATFGVYSPVALSKYGIDVPVMNLGLGVERLAMISGNFADVREMVYPQFYEHKLNDRNVASMVKLDKVPVMDEIYDLTKELIESCVKNKDLKSPCELAIEKTFSFGKTKKNVKINIFEKEEGKNLLGPSILNEIYVYDGNVIGIPESFDGVKEEFKDFLEKGKSEGVATGIRYIDALCFKITSKLEEAFVSNTTEFKVKVPIVRSLSDINLKIDDIALKQIMSKNKVIDVRGPVFLNVEVKIE

SEQ ID NO: 12 - DNA, 24 bp, synthetic construct
  source 1..24: mol_type = other DNA
cgctttgaggaatcccatatgggg

SEQ ID NO: 13 - DNA, 32 bp, synthetic construct
  source 1..32: mol_type = other DNA
gaaactgcagttaatggtgatgatgatggtgc

SEQ ID NO: 14 - DNA, 43 bp, synthetic construct
  source 1..43: mol_type = other DNA
cgtaagaagacccttaaaannknnkgtcgtaaacgaacgaatc

SEQ ID NO: 15 - DNA, 30 bp, synthetic construct
  source 1..30: mol_type = other DNA
cgttagaagacttttaaggtataggcaccg

SEQ ID NO: 16 - DNA, 40 bp, synthetic construct
  source 1..40: mol_type = other DNA
cgaatgaagacatgtggccnnkgcaggctggtgtgctgac

SEQ ID NO: 17 - DNA, 37 bp, synthetic construct
  source 1..37: mol_type = other DNA
gcatagaagacggccacatcaaaagtaccctggtgac

SEQ ID NO: 18 - DNA, 38 bp, synthetic construct
  source 1..38: mol_type = other DNA
gatatgaagactttcgaacnnktcgatgaataccgcgc

SEQ ID NO: 19 - DNA, 30 bp, synthetic construct
  source 1..30: mol_type = other DNA
gcttagaagacgttcgaaagcatggtgttc

SEQ ID NO: 20 - DNA, 73 bp, synthetic construct
  source 1..73: mol_type = other DNA
tacacatgctggttaataccagtaattataatgagggagtccaaaaaacaatgaccaacatcaccaagagaag

SEQ ID NO: 21 - DNA, 73 bp, synthetic construct
  source 1..73: mol_type = other DNA
aaaatcagacaccgtggagcaggacactcctgccccacgtattgccattacttcacaatgtacatattccggg

SEQ ID NO: 22 - DNA, 18 bp, synthetic construct
  source 1..18: mol_type = other DNA
tacaacgaaccaacttcc

SEQ ID NO: 23 - DNA, 20 bp, synthetic construct
  source 1..20: mol_type = other DNA
acgggccacatcaaaagtac

SEQ ID NO: 24 - DNA, 36 bp, synthetic construct
  source 1..36: mol_type = other DNA
gcaggctggtgtgctgcttacaacgaaccaacttcc

SEQ ID NO: 25 - DNA, 21 bp, synthetic construct
  source 1..21: mol_type = other DNA
agcagcacaccagcctgcacg

SEQ ID NO: 26 - DNA, 18 bp, synthetic construct
  source 1..18: mol_type = other DNA
gcaggctggtgtgctgac

SEQ ID NO: 27 - DNA, 18 bp, synthetic construct
  source 1..18: mol_type = other DNA
ctggtgacgggtgtcgag

SEQ ID NO: 28 - DNA, 37 bp, synthetic construct
  source 1..37: mol_type = other DNA
ggtacttttgatgtggccgcggcaggctggtgtgctg

SEQ ID NO: 29 - DNA, 25 bp, synthetic construct
  source 1..25: mol_type = other DNA
cgcggccacatcaaaagtaccctgg

SEQ ID NO: 30 - protein, 247 aa, synthetic construct
MPSKGEELFTGVVPILVELDGDVNGHKFSVRGEGEGDATNGKLTLKFICTTGKLPVPWPTLVTTLTYGVQCFSRYPDHMKRHDFFKSAMPEGYVQERTISFKDDGTYKTRAEVKFEGDTLVNRIELKGIDFKEDGNILGHKLEYNFNSHXVYITADKQKNGIKANFKIRHNVEDGSVQLADHYQQNTPIGDGPVLLPDNHYLSTQSVLSKDPNEKRDHMVLLEFVTAAGITHGMDELYKGSHHHHHH

SEQ ID NO: 31 - protein, 82 aa, synthetic construct
MQIFVKTLTGKTITLEVEPSDTIENVKAKIQDKEGIPPDQQRLIFAGKQLEDGRTLSDYNIQXESTLHLVLRLRGGHHHHHH

SEQ ID NO: 32 - protein, 146 aa, synthetic construct
MKYLLPTAAAGLLLLAAQPAMAQVQLVESGGALVQPGGSLRLSCAASGFPVNRYSMRWYRQAPGKEREWVAGMSSAGDRSSYEDSVKGRFTISRDDARNTVYLQMNSLKPEDTAVYYCNVNVGFEYWGQGTQVTVSSKKKHHHHHH

SEQ ID NO: 33 - protein, 146 aa, synthetic construct
MKYLLPTAAAGLLLLAAQPAMAQVQLVESGGALVQPGGSLXLSCAASGFPVNRYSMRWYRQAPGKEREWVAGMSSAGDRSSYEDSVKGRFTISRDDARNTVYLQMNSLKPEDTAVYYCNVNVGFEYWGQGTQVTVSSKKKHHHHHH

SEQ ID NO: 34 - protein, 146 aa, synthetic construct
MKYLLPTAAAGLLLLAAQPAMAQVQLVESGGALVQPGGSLRLSCAASGFPVNRYSMRWYRQAPGKEREWVAGMSSAGDRSSYEDSVKGRFTISRDDAXNTVYLQMNSLKPEDTAVYYCNVNVGFEYWGQGTQVTVSSKKKHHHHHH

SEQ ID NO: 35 - protein, 224 aa, synthetic construct
MSPILGYWKIKGLVQPTRLLLEYLEEKYEEHLYERDEGDKWRNKKFELGLXFPNLPYYIDGDVKLTQSMAIIRYIADKHNMLGGCPKERAEISMLEGAVLDIRYGVSRIAYSKDFETLKVDFLSKLPEMLKMFEDRLCHKTYLNGDHVTHPDFMLYDALDVVLYMDPMCLDAFPKLVCFKKRIEAIPQIDKYLKSSKYIAWPLQGWQATFGGGDHPPKHHHHHH

SEQ ID NO: 36 - protein, 99 aa, synthetic construct
MENLLEVLFQGPGGGGSMQIFVKTLTGKTITLEVEPSDTIENVKAKIQDKEGIPPDQQRLIFAGKQLEDGRTLSDYNIQXESTLHLVLRLRGGHHHHHH

SEQ ID NO: 37 - protein, 549 aa, synthetic construct
MGTNITKRSLVAAGVLAALMAGNVALAADVPAGVTLAEKQTLVRNNGSEVQSLDPHKIEGVPESNISRDLFEGLLVSDLDGHPAPGVAESWDNKDAKVWTFHLRKDAKWSDGTPVTAQDFVYSWQRSVDPNTASPYASYLQYGHIAGIDEILEGKKPITDLGVKAIDDHTLEVTLSEPVPYFYKLLVHPSTSPVPKAAIEKFGEKWTQPGNIVTNGAYTLKDWVVNERIVLERSPTYWNNAKTVINQVTYLPIASEVTDVNRYRSGEIDMTNNSMPIELFQKLKKEIPDEVHVDPYLCTYYYEINNQKPPFNDVRVRTALKLGMDRDIIVNKVKAQGNMPAYGYTPPYTDGAKLTQPEWFGWSQEKRNEEAKKLLAEAGYTADKPLTINLLYNTSDLHKKLAIAASSLWKKNIGVNVKLVNQEWKTFLDTRHQGTFDVARAGWCADYNEPTSFLNTMLSNSSMNTAHYKSPAFDSIMAETLKVTDEAQRTALYTKAEQQLDKDSAIVPVYYYVNARLVKPWVGGYTGKDPLDNTYTRNMYIVKHHHHHH

SEQ ID NO: 38 - protein, 549 aa, synthetic construct
MGTNITKRSLVAAGVLAALMAGNVALAADVPAGVTLAEKQTLVRNNGSEVQSLDPHKIEGVPESNISRDLFEGLLVSDLDGHPAPGVAESWDNKDAKVWTFHLRKDAKWSDGTPVTAQDFVYSWQRSVDPNTASPYASYLQYGHIAGIDEILEGKKPITDLGVKAIDDHTLEVTLSEPVPYFYKLLVHPSTSPAPKAAIEKFGEKWTQPGNIVTNGAYTLKLAVVNERIVLERSPTYWNNAKTVINQVTYLPIASEVTDVNRYRSGEIDMTNNSMPIELFQKLKKEIPDEVHVDPYLCTYYYEVNNQKPPFNDVRVRTALKLGMDRDIIVNKVKAQGDMPAYGYTPPYTDGAKLTQPEWFGWSQEKRNEEAKKLLAEAGYTADKPLTINLLYNTSDLHKKLAIAASSLWKKNIGVNVKLVNQEWKTFLDTRHQGTFDVAQAGWCADYNEPTSFLNTMLSNHSMNTAHYKSPAFDSIMAETLKVTDEAQRTALYTKAEQQLDKDSAIVPVYYYVNARLVKPWVGGYTGKDPLDNTYTRNMYIVKHHHHHH

SEQ ID NO: 39 - protein, 280 aa, synthetic construct
MGADLADRFAELERRYDARLGVYVPATGTTAAIEYRADERFAFCSTFKAPLVAAVLHQNPLTHLDKLITYTSDDIRSISPVAQQHVQTGMTIGQLCDAAIRYSDGTAANLLLADLGGPGGGTAAFTGYLRSLGDTVSRLDAEEPELNRDPPGDERDTTTPHAIALVLQQLVLGNALPPDKRALLTDWMARNTTGAKRIRAGFPADWKVIDKTGTGDYGRANDIAVVWSPTGVPYVVAVMSDRAGGGYDAEPREALLAEAATCVAGVLAGSGGSGHHHHHH

SEQ ID NO: 40 - protein, 280 aa, synthetic construct
MGADLADRFAELERRYDARLGVYVPATGTTAAIEYRADERFAFCSTFKAPLVAAVLHQNPLTHLDKLITYTSDDIRSISPVAQQHVQTGMTIGQLCDAAIRYSDGTAANLLLADLGGPGGGTAAFTGYLRSLGDTVSRLDAEEPELNRDPPGDERDTTTPHAIALVLQQLVLGNALPPDKRALLTDWMARNTTGAXRIRAGFPADWKVIDKTGTGDYGRANDIAVVWSPTGVPYVVAVMSDRAGGGYDAEPREALLAEAATCVAGVLAGSGGSGHHHHHH

SEQ ID NO: 41 - protein, 99 aa, synthetic construct
MADEKPKEGVKTENNDHINLKVAGQDGSVVQFKIKRHTPLSKLMKAYCERQGLSMRQIRFRFDGQPINETDTPAQLEMEDEDTIDVFQQQTGGHHHHHH

SEQ ID NO: 42 - protein, 99 aa, synthetic construct
MADEKPKEGVKTENNDHINLKVAGQDGSVVQFKIKRHTPLSKLMXAYCERQGLSMRQIRFRFDGQPINETDTPAQLEMEDEDTIDVFQQQTGGHHHHHH

SEQ ID NO: 43 - protein, 179 aa, synthetic construct
MADQLTEEQIAEFKEAFSLFDKDGDGTITTKELGTVMRSLGQNPTEAELQDMINEVDADGNGTIDFPEFLTMMARKMKDTDSEEEIREAFRVFDKDGNGYISAAELRHVMTNLGEKLTDEEVDEMIREADIDGDGQVNYEEFVQMMTAKSAWSHPQFEKGGGSGGGSGGSAWSHPQFEK

SEQ ID NO: 44 - protein, 179 aa, synthetic construct
MADQLTEEQIAEFKEAFSLFDKDGDGTITTKELGTVMRSLXQNPTEAELQDMINEVDADGNGTIDFPEFLTMMARKMKDTDSEEEIREAFRVFDKDGNGYISAAELRHVMTNLGEKLTDEEVDEMIREADIDGDGQVNYEEFVQMMTAKSAWSHPQFEKGGGSGGGSGGSAWSHPQFEK

SEQ ID NO: 45 - protein, 144 aa, synthetic construct
MARTKQTARKSTGGKAPRKQLATKAARKSAPATGGVKKPHRYRPGTVALREIRRYQKSTELLIRKLPFQRLVREIAQDFKTDLRFQSSAVMALQEASEAYLVALFEDTNLCAIHAKRVTIMPKDIQLARRIRGERARSHHHHHH

SEQ ID NO: 46 - protein, 144 aa, synthetic construct
MARTKQTARKSTGGKAPRKQLATKAARKSAPATGGVKKPHRYRPGTVALREIRRYQKSTELLIRKLPFQRLVREIAQDFKTDLRFQSSAVMALQEASEAYLVALFEDTNLCAIHAKRVTIMPXDIQLARRIRGERARSHHHHHH

SEQ ID NO: 47 - protein, 144 aa, synthetic construct
MARTKQTARKSTGGKAPRKQLATKAARKSAPATGGVKKPHRYRPGTVALREIRRYQKSTELLIRKLPFQRLVREIAQDFXTDLRFQSSAVMALQEASEAYLVALFEDTNLCAIHAKRVTIMPXDIQLARRIRGERARSHHHHHH

SEQ ID NO: 48 - protein, 144 aa, synthetic construct
MARTKQTARKSTGGKAPRKQLATKAARXSAPATGGVKKPHRYRPGTVALREIRRYQKSTELLIRKLPFQRLVREIAQDFXTDLRFQSSAVMALQEASEAYLVALFEDTNLCAIHAKRVTIMPXDIQLARRIRGERARSHHHHHH

SEQ ID NO: 49 - protein, 305 aa, synthetic construct
MSNKYRVRKNVLHLTDTEKRDFVRTVLILKEKGIYDRYIAWHGAAGKFHTPPGSDRNAAHMSSAFLPWHREYLLRFERDLQSINPEVTLPYWEWETDAQMQDPSQSQIWSADFMGGNGNPIKDFIVDTGPFAAGRWTTIDEQGNPSGGLKRNFGATKEAPTLPTRDDVLNALKITQYDTPPWDMTSQNSFRNQLEGFINGPQLHNRVHRWVGGQMGVVPTAPNDPVFFLHHANVDRIWAVWQIIHRNQNYQPMKNGPFGQNFRDPMYPWNTTPEDVMNHRKLGYVYDIELRKSKRSSLEHHHHHH

SEQ ID NO: 50 - protein, 760 aa, synthetic construct
MASETFEFQAEITQLMSLIINTVYSNKEIFLRELISNASDALDKIRYKSLSDPKQLETEPDLFIRITPKPEQKVLEIRDSGIGMTKAELINNLGTIAKSGTKAFMEALSAGADVSMIGQFGVGFYSLFLVADRVQVISKSNDDEQYIWESNAGGSFTVTLDEVNERIGRGTILRLFLKDDQLEYLEEKRIKEVIKRHSEFVAYPIQLVVTKEVEKEVPIPEEEKKDEEKKDEEKKDEDDKKPKLEEVDEEEEKKPKTKKVKEEVQEIEELNKTKPLWTRNPSDITQEEYNAFYKSISNDWEDPLYVKHFSVEGQLEFRAILFIPKRAPFDLFESKKKKNNIKLYVRRVFITDEAEDLIPEWLSFVKGVVDSEDLPLNLSREMLQQNKIMKVIRKNIVKKLIEAFNEIAEDSEQFEKFYSAFSKNIKLGVHEDTQNRAALAKLLRYNSTKSVDELTSLTDYVTRMPEHQKNIYYITGESLKAVEKSPFLDALKAKNFEVLFLTDPIDEYAFTQLKEFEGKTLVDITKDFELEETDEEKAEREKEIKEYEPLTKALKEILGDQVEKVVVSYKLLDAPAAIRTGQFGWSANMERIMKAQALRDSSMSSYMSSKKTFEISPKSPIIKELKKRVDEGGAQDKTVKDLTKLLYETALLTSGFSLDEPTSFASRINRLISLGLNIDEDEETETAPEASTAAPVEEVPADTEMEEVDPGEQKCEEWKRRYEKEKEKNARLKGKVEKLEIELARWRPGSAWSHHHHHHH

SEQ ID NO: 51 - protein, 760 aa, synthetic construct
MASETFEFQAEITQLMSLIINTVYSNKEIFLRELISNASDALDKIRYKSLSDPKQLETEPCLFIRITPKPEQKVLEIRDSGIGMTKAELINNLGTIAKSGTKAFMEALSAGADVSMIGQFGVGFYSLFLVADRVQVISKSNDDEQYIWESNAGGSFTVTLDEVNERIGRGTILRLFLKDDQLEYLEEKRIKEVIKRHSEFVAYPIQLVVTKEVEKEVPIPEEEKKDEEKKDEEKKDEDDKKPKLEEVDEEEEKKPKTKKVKEEVQEIEELNKTKPLWTRNPSDITQEEYNAFYKSISNDWEDPLYVKHFSVEGQLEFRAILFIPKRAPFDLFESKKKKNNIKLYVRRVFITDEAEDLIPEWLSFVKGVVDSEDLPLNLSREMLQQNKIMKVIRKNIVKKLIEAFNEIAEDSEQFEKFYSAFSKNIKLGVHEDTQNRAALAKLLRYNSTKSVXELTSLTDYVTRMPEHQKNIYYITGESLKAVEKSPFLDALKAKNFEVLFLTDPIDEYAFTQLKEFEGKTLVDITKDFELEETDEEKAEREKEIKEYEPLTKALKEILGDQVEKVVVSYKLLDAPAAIRTGQFGWSANMERIMKAQALRDSSMSSYMSSKKTFEISPKSPIIKELKKRVDEGGAQDKTVKDLTKLLYETALLTSGFSLDEPTSFASRINRLISLGLNIDEDEETETAPEASTAAPVEEVPADTEMEEVDPGEQKCEEWKRRYEKEKEKNARLKGKVEKLEIELARWRPGSAWSHHHHHHH

SEQ ID NO: 52 - protein, 419 aa, synthetic construct
MDKKPLDVLISATGLWMSRTGTLHKIKHHEVSRSKIYIEMACGDHLVVNNSRSCRTARAFRHHKYRKTCKRCRVSGEDINNFLTRSTESKNSVKVRVVSAPKVKKAMPKSVSRAPKPLENSVGAKASTNTSRSVPSPAKSTPNSSVPASAPAPSLTRSQLDRVEALLSPEDKISLNMAKPFRELEPELVTRRKNDFQRLYTNDREDYLGKLERDITKFFVDRGFLEIKSPILIPAEYVERMGINNDTELSKQIFRVDKNLCLRPMMAPTIFNYARKLDRILPGPIKIFEVGPCYRKESDGKEHLEEFTMVNFFQMGSGCTRENLEALIKEFLDYLEIDFEIVGDSCMVYGDTLDIMHGDLELSSAVVGPVSLDREWGIDKPWIGAGFGLERLLKVMHGFKNIKRASRSESYYNGISTNL

SEQ ID NO: 53 - protein, 247 aa, synthetic construct
MPSKGEELFTGVVPILVELDGDVNGHKFSVRGEGEGDATXGKLTLKFICTTGKLPVPWPTLVTTLTYGVQCFSRYPDHMKRHDFFKSAMPEGYVQERTISFKDDGTYKTRAEVKFEGDTLVNRIELKGIDFKEDGNILGHKLEYNFNSHXVYITADKQKNGIKANFKIRHNVEDGSVQLADHYQQNTPIGDGPVLLPDNHYLSTQSVLSKDPNEKRDHMVLLEFVTAAGITHGMDELYKGSHHHHHH

SEQ ID NO: 54 - protein, 184 aa, synthetic construct
MQIFVKTLTGKTITLEVEPSDTIENVKAKIQDKEGIPPDQQRLIFAGXQLEDGRTLSDYNIQKESTLHLVLRLRGGEDLYFQSMADEKPKEGVKTENNDHINLXVAGQDGSVVQFKIKRHTPLSKLMKAYCERQGLSMRQIRFRFDGQPINETDTPAQLEMEDEDTIDVFQQQQNGLHHHHHHH

SEQ ID NO: 55 - protein, 503 aa, synthetic construct
MEFSVKSGSPEKQRSACIVVGVFEPRRLSPIAEQLDKISDGYISALLRRGELEGKPGQTLLLHHVPNVLSERILLIGCGKERELDERQYKQVIQKTINTLNDTGSMEAVCFLTELHVKGRNNYWKVRQAVETAKETLYSFDQLKTNKSEPRRPLRKMVFNVPTRRELTSGERAIQHGLAIAAGIKAAKDLGNMPPNICNAAYLASQARQLADSYSKNVITRVIGEQQMKELGMHSYLAVGQGSQNESLMSVIEYKGNASEDARPIVLVGKGLTFDSGGISIKPSEGMDEMKYDMCGAAAVYGVMRMVAELQLPINVIGVLAGCENMPGGRAYRPGDVLTTMSGQTVEVLNTDAEGRLVLCDVLTYVERFEPEAVIDVATLTGACVIALGHHITGLMANHNPLAHELIAASEQSGDRAWRLPLGDEYQEQLESNFADMANIGGRPGGAITAGCFLSRFTRKYNWAHLDIAGTAWRSGKAKGATGRPVALLAQFLLNRAGFNGEE

SEQ ID NO: 56 - protein, 427 aa, synthetic construct
MTEAMKITLSTQPADARWGEKATYSINNDGITLHLNGADDLGLIQRAARKIDGLGIKHVQLSGEGWDADRCWAFWQGYKAPKGTRKVVWPDLDDAQRQELDNRLMIIDWVRDTINAPAEELGPSQLAQRAVDLISNVAGDRVTYRITKGEDLREQGYMGLHTVGRGSERSPVLLALDYNPTGDKEAPVYACLVGKGITFDSGGYSIKQTAFMDSMKSDMGGAATVTGALAFAITRGLNKRVKLFLCCADNLISGNAFKLGDIITYRNGKKVEVMNTDAEGRLVLADGLIDASAQKPEMIIDAATLTGAAKTALGNDYHALFSFDDALAGRLLASAAQENEPFWRLPLAEFHRSQLPSNFAELNNTGSAAYPAGASTAAGFLSHFVENYQQGWLHIDCSATYRKAPVEQWSAGATGLGVRTIANLLTA

SEQ ID NO: 57 - protein, 408 aa, synthetic construct
MDKLLERFLNYVSLDTQSKAGVRQVPSTEGQWKLLHLLKEQLEEMGLINVTLSEKGTLMATLPANVPGDIPAIGFISHVDTSPDCSGKNVNPQIVENYRGGDIALGIGDEVLSPVMFPVLHQLLGQTLITTDGKTLLGADDKAGIAEIMTALAVLQQKKIPHGDIRVAFTPDEEVGKGAKHFDVDAFDARWAYTVDGGGVGELEFENFNAASVNIKIVGNNVHPGTAKGVMVNALSLAARIHAEVPADESPEMTEGYEGFYHLASMKGTVERADMHYIIRDFDRKQFEARKRKMMEIAKKVGKGLHPDCYIELVIEDSYYNMREKVVEHPHILDIAQQAMRDCDIEPELKPIRGGTDGAQLSFMGLPCPNLFTGGYNYHGKHEFVTLEGMEKAVQVIVRIAELTAQRK

SEQ ID NO: 58 - protein, 870 aa, synthetic construct
MTQQPQAKYRHDYRAPDYQITDIDLTFDLDAQKTVVTAVSQAVRHGASDAPLRLNGEDLKLVSVHINDEPWTAWKEEEGALVISNLPERFTLKIINEISPAANTALEGLYQSGDALCTQCEAEGFRHITYYLDRPDVLARFTTKIIADKIKYPFLLSNGNRVAQGELENGRHWVQWQDPFPKPCYLFALVAGDFDVLRDTFTTRSGREVALELYVDRGNLDRAPWAMTSLKNSMKWDEERFGLEYDLDIYMIVAVDFFNMGAMENKGLNIFNSKYVLARTDTATDKDYLDIERVIGHEYFHNWTGNRVTCRDWFQLSLKEGLTVFRDQEFSSDLGSRAVNRINNVRTMRGLQFAEDASPMAHPIRPDMVIEMNNFYTLTVYEKGAEVIRMIHTLLGEENFQKGMQLYFERHDGSAATCDDFVQAMEDASNVDLSHFRRWYSQSGTPIVTVKDDYNPETEQYTLTISQRTPATPDQAEKQPLHIPFAIELYDNEGKVIPLQKGGHPVNSVLNVTQAEQTFVFDNVYFQPVPALLCEFSAPVKLEYKWSDQQLTFLMRHARNDFSRWDAAQSLLATYIKLNVARHQQGQPLSLPVHVADAFRAVLLDEKIDPALAAEILTLPSVNEMAELFDIIDPIAIAEVREALTRTLATELADELLAIYNANYQSEYRVEHEDIAKRTLRNACLRFLAFGETHLADVLVSKQFHEANNMTDALAALSAAVAAQLPCRDALMQEYDDKWHQNGLVMDKWFILQATSPAANVLETVRGLLQHRSFTMSNPNRIRSLIGAFAGSNPAAFHAEDGSGYLFLVEMLTDLNSRNPQVASRLIEPLIRLKRYDAKRQEKMRAALEQLKGLENLSGDLYEKITKALA

SEQ ID NO: 59 - protein, 193 aa, synthetic construct
MSDTTELVDLAVIFPDLEIELKYACADNITGKAIYQQARCLLHKDAITALAKSISIAQLSGLQLVIYDAYRPQQAQAMLWQACPDPQYVVDVTVGSNHSRGTAIDLTLRDEHGNILDMGAGFDEMHERSHAYHPSVPPAAQRNRLLLNAIMTGGGFVGISSEWWHFELPQAASYPLLADQFSCFISPGTQHVS

SEQ ID NO: 60 - protein, 345 aa, synthetic construct
MDLSLLKALSEADAIASSEQEVRQILLEEADRLQKEVRFDGLGSVLIRLNESTGPKVMICAHMDEVGFMVRSISREGAIDVLPVGNVRMAARQLQPVRITTREECKIPGLLDGDRQGNDVSAMRVDIGARSYDEVMQAGIRPGDRVTFDTTFQVLPHQRVMGKAFDDRLGCYLLVTLLRELHDAELPAEVWLVASSSEEVGLRGGQTATRAVSPDVAIVLDTACWAKNFDYGAANHRQIGNGPMLVLSDKSLIAPPKLTAWVETVAAEIGVPLQADMFSNGGTDGGAVHLTGTGVPTVVMGPATRHGHCAASIADCRDILQMQQLLSALIQRLTRETVVQLTDFR

SEQ ID NO: 61 - protein, 360 aa, synthetic construct
MTLLASLRDWLKAQQLDAVLLSSRQNKQPHLGISTGSGYVVISRESAHILVDSRYYVEVEARAQGYQLHLLDATNTLTTIVNQIIADEQLQTLGFEGQQVSWETAHRWQSELNAKLVSATPDVLRQIKTPEEVEKIRLACGIADRGAEHIRRFIQAGMSEREIAAELEWFMRQQGAEKASFDTIVASGWRGALPHGKASDKIVAAGEFVTLDFGALYQGYCSDMTRTLLVNGEGVSAESHLLFNVYQIVLQAQLAAISAIRPGVRCQQVDDAARRVITEAGYGDYFGHNTGHAIGIEVHEDPRFSPRDTTTLQPGMLLTVEPGIYLPGQGGVRIEDVVLVTPQGAEVLYAMPKTVLLTGE

SEQ ID NO: 62 - protein, 356 aa, synthetic construct
MNIELLQQLCEASAVSGDEQEVRDILINTLEPCVNEITFDGLGSFVARKGNKGPKVAVVGHMDEVGFMVTHIDESGFLRFTTIGGWWNQSMLNHRVTIRTHKGVKIPGVIGSVAPHALTEKQKQQPLSFDEMFIDIGANSREEVEKRGVEIGNFISPEANFACWGEDKVVGKALDNRIGCAMMAELLQTVNNPEITLYGVGSVEEEVGLRGAQTSAEHIKPDVVIVLDTAVAGDVPGIDNIKYPLKLGQGPGLMLFDKRYFPNQKLVAALKSCAAHNDLPLQFSTMKTGATDGGRYNVMGGGRPVVALCLPTRYLHANSGMISKADYEALLTLIRGFLTTLTAEKVNAFSQFRQVD

SEQ ID NO: 63 - protein, 373 aa, synthetic construct
MSFSVQETLFSLLQHNAISGHENAVADVMLCEFRRQAKEVWRDRLGNVVARYGSDKPDALRLMIFAHMDEVGFMVRKIEPSGFLRFERVGGPAQVTMAGSIVTLTGDKGPVMGCIGIKSYHFAKGDERTQSPSVDKLWIDIGAKDKDDAIRMGIQVGTPVTLYNPPQLLANDLVCSKALDDRLGCTALLGVADAISTMELDIAVYLVASVQEEFNIRGIVPVLRRVKPDLAIGIDITPSCDTPDLHDYSEVRINQGVGITCLNYHGRGTLAGLITPPRLIRMLEQTALEHNIPVQREVAPGVITETGYIQVEQDGIPCASLSIPCRYTHSPAEVASLRDLTDCIRLLTALAGMSAAHFPVEPDSGTTQEAHPL

SEQ ID NO: 64 - protein, 489 aa, synthetic construct [sequence omitted]